European Patent Application EP 4 541 817 A2, published April 23, 2025. Title: Nucelic acid molecule coding CAR, CAR, immunocyte comprising CAR, pharmaceutical composition comprising the immunocyte, method for improving cytotoxic activity and method for producing imunnocyte comprising CAR. Applicant: MIE UNIVERSITY. The sequence listing filed with the application follows.

SEQUENCE LISTING (120 sequences)

SEQ ID NO: 1 - protein, 10 aa, synthetic construct
GVYDGREHTV

SEQ ID NO: 2 - protein, 9 aa, synthetic construct
LYVDSLFFL

SEQ ID NO: 3 - DNA, 21 bp, synthetic construct
  source 1..21: mol_type = other DNA
ggaggcaccttcagcagctat

SEQ ID NO: 4 - DNA, 12 bp, synthetic construct
  source 1..12: mol_type = other DNA
cctatctttggt

SEQ ID NO: 5 - DNA, 30 bp, synthetic construct
  source 1..30: mol_type = other DNA
ccccggcgggcatatcatgatgcttttgat

SEQ ID NO: 6 - DNA, 24 bp, synthetic construct
  source 1..24: mol_type = other DNA
ggagaccatattggaagtaaaagt

SEQ ID NO: 7 - DNA, 18 bp, synthetic construct
  source 1..18: mol_type = other DNA
tgggacagcagcactgcg

SEQ ID NO: 8 - DNA, 723 bp, synthetic construct
  source 1..723: mol_type = other DNA
cagctggtacagtctggggctgaggtgaagaagcctgggtcctcggtgaaggtctcctgcaaggcttctggaggcaccttcagcagctatgctatcagctgggtgcgacaggcccctggacaagggcttgagtggatgggagggatcatccctatctttggtacagcaaactacgcacagaagttccagggcagagtcacgattaccgcggacaaatccacgagcacagcctacatggagctgagcagcctgagatctgaggacacggccgtgtattactgtgcgagatccccccggcgggcatatcatgatgcttttgatatctggggccaagggacaatggtcaccgtctcttcaggtggaggcggttcaggcggaggtggcagcggcggtggcgggagttcctatgagctgactcagccaccctcgatgtcagtggccccaggaaagacggccagcattacctgtggcggagaccatattggaagtaaaagtgttcactggtaccagcagaagccaggccaggcccctgtactggtcgtctatgatgatagcgaccggccctcagggatccctgagcgattctctggctccaactctgggaacacagccactctgaccatcagcgggacccaggctatggatgaggctgactattactgtctggcgtgggacagcagcactgcgatcttcggcggaggcacccagctgaccgtcctcgtg

SEQ ID NO: 9 - DNA, 723 bp, synthetic construct
  source 1..723: mol_type = other DNA
cagctggtacagtctggggctgaggtgaagaagcctgggtcctcggtgaaggtctcctgcaaggcttctggaggcaccttcagcagctatgctatcagctgggtgcgacaggcccctggacaagggcttgagtggatgggagggatcatccctatctttggtacagcaaactacgcacagaagttccagggcagagtcacgattaccgcggacaaatccacgagcacagcctacatggagctgagcagcctgagatctgaggacacggccgtgtattactgtgcgagatccccccggcgggcatatcatgatgcttttgatatctggggccaagggacaatggtcaccgtctcttcaggtggaggcggttcaggcggaggtggcagcggcggtggcgggagttcctatgagctgactcagccaccctcgatgtcagtggccccaggaaagacggccagcattacctgtggcggagaccatattggaagtaaaagtgttcactggtaccagcagaagccaggccaggcccctgtactggtcgtctatgatgatagcgaccggccctcagggatccctgagcgattcgagggcgagaacgaggggaacgaggccactctgaccatcagcgggacccaggctatggatgaggctgactattactgtctggcgtgggacagcagcactgcgatcttcggcggaggcacccagctgaccgtcctcgtg

SEQ ID NO: 10 - DNA, 723 bp, synthetic construct
  source 1..723: mol_type = other DNA
cagctggtacagtctggggctgaggtgaagaagcctgggtcctcggtgaaggtctcctgcaaggcttctggaggcaccttcagcagctatgctatcagctgggtgcgacaggcccctggacaagggcttgagtggatgggagggatcatccctatctttggtacagcaaactacgcacagaagttccagggcagagtcacgattaccgcggacaaatccacgagcacagcctacatggagctgagcagcctgagatctgaggacacggccgtgtattactgtgcgagatccccccggcgggcatatcatgatgcttttgatatctggggccaagggacaatggtcaccgtctcttcaggtggaggcggttcaggcggaggtggcagcggcggtggcgggagttcctatgagctgactcagccaccctcgatgtcagtggccccaggaaagacggccagcattacctgtggcggagaccatattggaagtaaaagtgttcactggtaccagcagaagccaggccaggcccctgtactggtcgtctatgatgatagcgaccggccctcagggatccctgagcgattcgagggcgagaacgaggggaacacagccgagctgaccatcagcgggacccaggctatggatgaggctgactattactgtctggcgtgggacagcagcactgcgatcttcggcggaggcacccagctgaccgtcctcgtg

SEQ ID NO: 11 - DNA, 723 bp, synthetic construct
  source 1..723: mol_type = other DNA
cagctggtacagtctggggctgaggtgaagaagcctgggtcctcggtgaaggtctcctgcaaggcttctggaggcaccttcagcagctatgctatcagctgggtgcgacaggcccctggacaagggcttgagtggatgggagggatcatccctatctttggtacagcaaactacgcacagaagttccagggcagagtcacgattaccgcggacaaatccacgagcacagcctacatggagctgagcagcctgagatctgaggacacggccgtgtattactgtgcgagatccccccggcgggcatatcatgatgcttttgatatctggggccaagggacaatggtcaccgtctcttcaggtggaggcggttcaggcggaggtggcagcggcggtggcgggagttcctatgagctgactcagccaccctcgatgtcagtggccccaggaaagacggccagcattacctgtggcggagaccatattggaagtaaaagtgttcactggtaccagcagaagccaggccaggcccctgtactggtcgtctatgatgatagcgaccggccctcagggatccctgagcgattctctggcgagaacgaggggaacgaggccgagctgaccatcagcgggacccaggctatggatgaggctgactattactgtctggcgtgggacagcagcactgcgatcttcggcggaggcacccagctgaccgtcctcgtg

SEQ ID NO: 12 - DNA, 723 bp, synthetic construct
  source 1..723: mol_type = other DNA
cagctggtacagtctggggctgaggtgaagaagcctgggtcctcggtgaaggtctcctgcaaggcttctggaggcaccttcagcagctatgctatcagctgggtgcgacaggcccctggacaagggcttgagtggatgggagggatcatccctatctttggtacagcaaactacgcacagaagttccagggcagagtcacgattaccgcggacaaatccacgagcacagcctacatggagctgagcagcctgagatctgaggacacggccgtgtattactgtgcgagatccccccggcgggcatatcatgatgcttttgatatctggggccaagggacaatggtcaccgtctcttcaggtggaggcggttcaggcggaggtggcagcggcggtggcgggagttcctatgagctgactcagccaccctcgatgtcagtggccccaggaaagacggccagcattacctgtggcggagaccatattggaagtaaaagtgttcactggtaccagcagaagccaggccaggcccctgtactggtcgtctatgatgatagcgaccggccatcagggatccctgagcgattcgaaggctccaactctgggaacgaggccgaactgaccatcagcgggacccaggctatggatgaggctgactattactgtctggcgtgggacagcagcactgcgatcttcggcggaggcacccagctgaccgtcctcgtg

SEQ ID NO: 13 - DNA, 723 bp, synthetic construct
  source 1..723: mol_type = other DNA
cagctggtacagtctggggctgaggtgaagaagcctgggtcctcggtgaaggtctcctgcaaggcttctggaggcaccttcagcagctatgctatcagctgggtgcgacaggcccctggacaagggcttgagtggatgggagggatcatccctatctttggtacagcaaactacgcacagaagttccagggcagagtcacgattaccgcggacaaatccacgagcacagcctacatggagctgagcagcctgagatctgaggacacggccgtgtattactgtgcgagatccccccggcgggcatatcatgatgcttttgatatctggggccaagggacaatggtcaccgtctcttcaggtggaggcggttcaggcggaggtggcagcggcggtggcgggagttcctatgagctgactcagccaccctcgatgtcagtggccccaggaaagacggccagcattacctgtggcggagaccatattggaagtaaaagtgttcactggtaccagcagaagccaggccaggcccctgtactggtcgtctatgatgatagcgaccggccatcagggatccctgaccgattctctggctccaactctgggaacacagccactctggacatcgacgggacccaggctatggatgaggctgactattactgtctggcgtgggacagcagcactgcgatcttcggcggaggcacccagctgaccgtcctcgtg

SEQ ID NO: 14 - DNA, 21 bp, synthetic construct
  source 1..21: mol_type = other DNA
ggggtttccctccccgactac

SEQ ID NO: 15 - DNA, 30 bp, synthetic construct
  source 1..30: mol_type = other DNA
tattactacggcggatcttatgcgatggac

SEQ ID NO: 16 - DNA, 18 bp, synthetic construct
  source 1..18: mol_type = other DNA
caggatataagcaaatac

SEQ ID NO: 17 - DNA, 18 bp, synthetic construct
  source 1..18: mol_type = other DNA
gggaataccctcccgtat

SEQ ID NO: 18 - DNA, 726 bp, synthetic construct
  source 1..726: mol_type = other DNA
gacatccaaatgacgcagactacaagcagcttgtcagcctcactgggagatcgagtcaccattagctgcagagctagccaggatataagcaaatacctgaactggtatcagcagaaacccgatggcaccgtgaagctgctgatctatcacacatctcggctgcatagtggagttccttctcgattttcaggctctggctctgggacagattatagtctgacaatctccaacttggaacaggaggatatagccacctatttctgccagcaagggaataccctcccgtatacatttggaggcggcactaagctggagattacgggtggaggcggttcaggcggaggtggcagcggcggtggcgggagtgaagtgaaactgcaggagtcaggcccaggccttgtcgcaccctcccaatccctgagtgtcacatgcacagtaagcggggtttccctccccgactacggtgtttcatggatcagacagcctccaaggaaaggacttgagtggctcggggtgatttggggtagcgaaaccacctactacaatagcgcgttgaagtccaggctcaccatcatcaaggataacagtaaatcccaggttttcctgaaaatgaatagcctgcagacagatgatactgccatatactactgcgccaaacactattactacggcggatcttatgcgatggactattggggtcaaggtacatctgtaaccgtgagttcc

SEQ ID NO: 19 - DNA, 726 bp, synthetic construct
  source 1..726: mol_type = other DNA
gacatccaaatgacgcagactacaagcagcttgtcagcctcactgggagatcgagtcaccattagctgcagagctagccaggatataagcaaatacctgaactggtatcagcagaaacccgatggcaccgtgaagctgctgatctatcacacatctcggctgcatagtggagttccttctcgattttcaggctctggcgaagggacagagtatgaactgacaatctccaacttggaacaggaggatatagccacctatttctgccagcaagggaataccctcccgtatacatttggaggcggcactaagctggagattacgggtggaggcggttcaggcggaggtggcagcggcggtggcgggagtgaagtgaaactgcaggagtcaggcccaggccttgtcgcaccctcccaatccctgagtgtcacatgcacagtaagcggggtttccctccccgactacggtgtttcatggatcagacagcctccaaggaaaggacttgagtggctcggggtgatttggggtagcgaaaccacctactacaatagcgcgttgaagtccaggctcaccatcatcaaggataacagtaaatcccaggttttcctgaaaatgaatagcctgcagacagatgatactgccatatactactgcgccaaacactattactacggcggatcttatgcgatggactattggggtcaaggtacatctgtaaccgtgagttcc

SEQ ID NO: 20 - DNA, 726 bp, synthetic construct
  source 1..726: mol_type = other DNA
gacatccaaatgacgcagactacaagcagcttgtcagcctcactgggagatcgagtcaccattagctgcagagctagccaggatataagcaaatacctgaactggtatcagcagaaacccgatggcaccgtgaagctgctgatctatcacacatctcggctgcatagtggagttccttctcgatttgatggcgatggcgatgggacagattatagtctgacaatctccaacttggaacaggaggatatagccacctatttctgccagcaagggaataccctcccgtatacatttggaggcggcactaagctggagattacgggtggaggcggttcaggcggaggtggcagcggcggtggcgggagtgaagtgaaactgcaggagtcaggcccaggccttgtcgcaccctcccaatccctgagtgtcacatgcacagtaagcggggtttccctccccgactacggtgtttcatggatcagacagcctccaaggaaaggacttgagtggctcggggtgatttggggtagcgaaaccacctactacaatagcgcgttgaagtccaggctcaccatcatcaaggataacagtaaatcccaggttttcctgaaaatgaatagcctgcagacagatgatactgccatatactactgcgccaaacactattactacggcggatcttatgcgatggactattggggtcaaggtacatctgtaaccgtgagttcc

SEQ ID NO: 21 - DNA, 726 bp, synthetic construct
  source 1..726: mol_type = other DNA
gacatccaaatgacgcagactacaagcagcttgtcagcctcactgggagatcgagtcaccattagctgcagagctagccaggatataagcaaatacctgaactggtatcagcagaaacccgatggcaccgtgaagctgctgatctatcacacatctcggctgcatagtggagttcctgaccgatttgatggcgatggctctgggacagattatagtctgacaatctccaacttggaacaggaggatatagccacctatttctgccagcaagggaataccctcccgtatacatttggaggcggcactaagctggagattacgggtggaggcggttcaggcggaggtggcagcggcggtggcgggagtgaagtgaaactgcaggagtcaggcccaggccttgtcgcaccctcccaatccctgagtgtcacatgcacagtaagcggggtttccctccccgactacggtgtttcatggatcagacagcctccaaggaaaggacttgagtggctcggggtgatttggggtagcgaaaccacctactacaatagcgcgttgaagtccaggctcaccatcatcaaggataacagtaaatcccaggttttcctgaaaatgaatagcctgcagacagatgatactgccatatactactgcgccaaacactattactacggcggatcttatgcgatggactattggggtcaaggtacatctgtaaccgtgagttcc

SEQ ID NO: 22 - DNA, 726 bp, synthetic construct
  source 1..726: mol_type = other DNA
gacatccaaatgacgcagactacaagcagcttgtcagcctcactgggagatcgagtcaccattagctgcagagctagccaggatataagcaaatacctgaactggtatcagcagaaacccgatggcaccgtgaagctgctgatctatcacacatctcggctgcatagtggagttccttctcgattttcaggctctggctctgggacagagtatgaactggagatctccaacttggaacaggaggatatagccacctatttctgccagcaagggaataccctcccgtatacatttggaggcggcactaagctggagattacgggtggaggcggttcaggcggaggtggcagcggcggtggcgggagtgaagtgaaactgcaggagtcaggcccaggccttgtcgcaccctcccaatccctgagtgtcacatgcacagtaagcggggtttccctccccgactacggtgtttcatggatcagacagcctccaaggaaaggacttgagtggctcggggtgatttggggtagcgaaaccacctactacaatagcgcgttgaagtccaggctcaccatcatcaaggataacagtaaatcccaggttttcctgaaaatgaatagcctgcagacagatgatactgccatatactactgcgccaaacactattactacggcggatcttatgcgatggactattggggtcaaggtacatctgtaaccgtgagttcc

SEQ ID NO: 23 - DNA, 726 bp, synthetic construct
  source 1..726: mol_type = other DNA
gacatccaaatgacgcagactacaagcagcttgtcagcctcactgggagatcgagtcaccattagctgcagagctagccaggatataagcaaatacctgaactggtatcagcagaaacccgatggcaccgtgaagctgctgatctatcacacatctcggctgcatagtggagttccttctcgatttgatggcgatggctctgggacagattatgatctgacaatctccaacttggaacaggaggatatagccacctatttctgccagcaagggaataccctcccgtatacatttggaggcggcactaagctggagattacgggtggaggcggttcaggcggaggtggcagcggcggtggcgggagtgaagtgaaactgcaggagtcaggcccaggccttgtcgcaccctcccaatccctgagtgtcacatgcacagtaagcggggtttccctccccgactacggtgtttcatggatcagacagcctccaaggaaaggacttgagtggctcggggtgatttggggtagcgaaaccacctactacaatagcgcgttgaagtccaggctcaccatcatcaaggataacagtaaatcccaggttttcctgaaaatgaatagcctgcagacagatgatactgccatatactactgcgccaaacactattactacggcggatcttatgcgatggactattggggtcaaggtacatctgtaaccgtgagttcc

SEQ ID NO: 24 - DNA, 726 bp, synthetic construct
  source 1..726: mol_type = other DNA
gacatccaaatgacgcagactacaagcagcttgtcagcctcactgggagatcgagtcaccattagctgcagagctagccaggatataagcaaatacctgaactggtatcagcagaaacccgatggcaccgtgaagctgctgatctatcacacatctcggctgcatagtggagttccttctcgatttgatggctctggcgatgggacagattatgatctgacaatctccaacttggaacaggaggatatagccacctatttctgccagcaagggaataccctcccgtatacatttggaggcggcactaagctggagattacgggtggaggcggttcaggcggaggtggcagcggcggtggcgggagtgaagtgaaactgcaggagtcaggcccaggccttgtcgcaccctcccaatccctgagtgtcacatgcacagtaagcggggtttccctccccgactacggtgtttcatggatcagacagcctccaaggaaaggacttgagtggctcggggtgatttggggtagcgaaaccacctactacaatagcgcgttgaagtccaggctcaccatcatcaaggataacagtaaatcccaggttttcctgaaaatgaatagcctgcagacagatgatactgccatatactactgcgccaaacactattactacggcggatcttatgcgatggactattggggtcaaggtacatctgtaaccgtgagttcc

SEQ ID NO: 25 - DNA, 726 bp, synthetic construct
  source 1..726: mol_type = other DNA
gacatccaaatgacgcagactacaagcagcttgtcagcctcactgggagatcgagtcaccattagctgcagagctagccaggatataagcaaatacctgaactggtatcagcagaaacccgatggcaccgtgaagctgctgatctatcacacatctcggctgcatagtggagttccttctcgatttgatggcgatggcgatgggacagattatgatctgacaatctccaacttggaacaggaggatatagccacctatttctgccagcaagggaataccctcccgtatacatttggaggcggcactaagctggagattacgggtggaggcggttcaggcggaggtggcagcggcggtggcgggagtgaagtgaaactgcaggagtcaggcccaggccttgtcgcaccctcccaatccctgagtgtcacatgcacagtaagcggggtttccctccccgactacggtgtttcatggatcagacagcctccaaggaaaggacttgagtggctcggggtgatttggggtagcgaaaccacctactacaatagcgcgttgaagtccaggctcaccatcatcaaggataacagtaaatcccaggttttcctgaaaatgaatagcctgcagacagatgatactgccatatactactgcgccaaacactattactacggcggatcttatgcgatggactattggggtcaaggtacatctgtaaccgtgagttcc

SEQ ID NO: 26 - DNA, 726 bp, synthetic construct
  source 1..726: mol_type = other DNA
gacatccaaatgacgcagactacaagcagcttgtcagcctcactgggagatcgagtcaccattagctgcagagctagccaggatataagcaaatacctgaactggtatcagcagaaacccgatggcaccgtgaagctgctgatctatcacacatctcggctgcatagtggagttccttctcgatttgaaggcgaaggcgaagggacagaatatgaactgacaatctccaacttggaacaggaggatatagccacctatttctgccagcaagggaataccctcccgtatacatttggaggcggcactaagctggagattacgggtggaggcggttcaggcggaggtggcagcggcggtggcgggagtgaagtgaaactgcaggagtcaggcccaggccttgtcgcaccctcccaatccctgagtgtcacatgcacagtaagcggggtttccctccccgactacggtgtttcatggatcagacagcctccaaggaaaggacttgagtggctcggggtgatttggggtagcgaaaccacctactacaatagcgcgttgaagtccaggctcaccatcatcaaggataacagtaaatcccaggttttcctgaaaatgaatagcctgcagacagatgatactgccatatactactgcgccaaacactattactacggcggatcttatgcgatggactattggggtcaaggtacatctgtaaccgtgagttcc

SEQ ID NO: 27 - protein, 5 aa, synthetic construct
GGGGS

SEQ ID NO: 28 - DNA, 69 bp, synthetic construct
  source 1..69: mol_type = other DNA
tacatttgggctccactggccggtacgtgtggggtccttctgctcagtctggtgatcactctgtattgc

SEQ ID NO: 29 - DNA, 84 bp, synthetic construct
  source 1..84: mol_type = other DNA
ttttgggtgctggtggtggttggtggagtcctggcttgctatagcttgctagtaacagtggcctttattattttctgggtgagg

SEQ ID NO: 30 - DNA, 318 bp, synthetic construct
  source 1..318: mol_type = other DNA
ggtcagcccaaggccaaccccactgtcactctgtttccgccctcctctgaggagctccaagccaacaaggccacactagtgtgtctgatcagtgacttctacccgggagctgtgacagtggcctggaaggcagatggcagccccgtcaaggcgggagtggagaccaccaaaccctccaaacagagcaacaacaagtacgcggccagcagctacctgagcctgacgcccgagcagtggaagtcccacagaagctacagctgccaggtcacgcatgaagggagcaccgtggagaagactgtggcccctacagaatgttcg

SEQ ID NO: 31 - DNA, 117 bp, synthetic construct
  source 1..117: mol_type = other DNA
atcgaagtgatgtaccctcctccttacctggacaacgagaagtccaacggcaccatcatccacgtgaagggcaagcacctgtgtccttctccactgttccccggacctagcaagcct

SEQ ID NO: 32 - DNA, 342 bp, synthetic construct
  source 1..342: mol_type = other DNA
ctgagagtgaagttcagcaggagcgcagacgcccccgcgtaccagcagggccagaaccagctctataacgagctcaatctaggacgaagagaggagtacgatgttttggacaagagacgtggccgggaccctgagatggggggaaagccgcagagaaggaagaaccctcaggaaggcctgtacaatgaactgcagaaagataagatggcggaggcctacagtgagattgggatgaaaggcgagcgccggaggggcaaggggcacgatggcctttaccagggtctcagtacagccaccaaggacacctacgacgcccttcacatgcaggccctgccccctcgc

SEQ ID NO: 33 - DNA, 123 bp, synthetic construct
  source 1..123: mol_type = other DNA
aaaagaggtcgtaagaagcttttgtacattttcaagcagccctttatgcggccggtgcaaacaactcaggaggaggatggatgtagctgtcggtttccagaggaagaggagggaggttgcgaa

SEQ ID NO: 34 - DNA, 120 bp, synthetic construct
  source 1..120: mol_type = other DNA
agtaagaggagcaggctcctgcacagtgactacatgaacatgactccccgccgccccgggcccacccgcaagcattaccagccctatgccccaccacgcgacttcgcagcctatcgctcc

SEQ ID NO: 35 - DNA, 147 bp, synthetic construct
  source 1..147: mol_type = other DNA
aggagtcagtgcatgtggccccgagagacccagctgctgctggaggtgccgccgtcgaccgaagacgccagaagctgccagttccccgaggaagagcggggcgagcgatcggcagaggagaaggggcggctgggagacctgtgggtg

SEQ ID NO: 36 - protein, 7 aa, synthetic construct
GGTFSSY

SEQ ID NO: 37 - protein, 4 aa, synthetic construct
PIFG

SEQ ID NO: 38 - protein, 10 aa, synthetic construct
PRRAYHDAFD

SEQ ID NO: 39 - protein, 8 aa, synthetic construct
GDHIGSKS

SEQ ID NO: 40 - protein, 6 aa, synthetic construct
WDSSTA

SEQ ID NO: 41 - protein, 241 aa, synthetic construct
QLVQSGAEVKKPGSSVKVSCKASGGTFSSYAISWVRQAPGQGLEWMGGIIPIFGTANYAQKFQGRVTITADKSTSTAYMELSSLRSEDTAVYYCARSPRRAYHDAFDIWGQGTMVTVSSGGGGSGGGGSGGGGSSYELTQPPSMSVAPGKTASITCGGDHIGSKSVHWYQQKPGQAPVLVVYDDSDRPSGIPERFSGSNSGNTATLTISGTQAMDEADYYCLAWDSSTAIFGGGTQLTVLV

SEQ ID NO: 42 - protein, 241 aa, synthetic construct
QLVQSGAEVKKPGSSVKVSCKASGGTFSSYAISWVRQAPGQGLEWMGGIIPIFGTANYAQKFQGRVTITADKSTSTAYMELSSLRSEDTAVYYCARSPRRAYHDAFDIWGQGTMVTVSSGGGGSGGGGSGGGGSSYELTQPPSMSVAPGKTASITCGGDHIGSKSVHWYQQKPGQAPVLVVYDDSDRPSGIPERFEGENEGNEATLTISGTQAMDEADYYCLAWDSSTAIFGGGTQLTVLV

SEQ ID NO: 43 - protein, 241 aa, synthetic construct
QLVQSGAEVKKPGSSVKVSCKASGGTFSSYAISWVRQAPGQGLEWMGGIIPIFGTANYAQKFQGRVTITADKSTSTAYMELSSLRSEDTAVYYCARSPRRAYHDAFDIWGQGTMVTVSSGGGGSGGGGSGGGGSSYELTQPPSMSVAPGKTASITCGGDHIGSKSVHWYQQKPGQAPVLVVYDDSDRPSGIPERFEGENEGNTAELTISGTQAMDEADYYCLAWDSSTAIFGGGTQLTVLV

SEQ ID NO: 44 - protein, 241 aa, synthetic construct
QLVQSGAEVKKPGSSVKVSCKASGGTFSSYAISWVRQAPGQGLEWMGGIIPIFGTANYAQKFQGRVTITADKSTSTAYMELSSLRSEDTAVYYCARSPRRAYHDAFDIWGQGTMVTVSSGGGGSGGGGSGGGGSSYELTQPPSMSVAPGKTASITCGGDHIGSKSVHWYQQKPGQAPVLVVYDDSDRPSGIPERFSGENEGNEAELTISGTQAMDEADYYCLAWDSSTAIFGGGTQLTVLV

SEQ ID NO: 45 - protein, 241 aa, synthetic construct
QLVQSGAEVKKPGSSVKVSCKASGGTFSSYAISWVRQAPGQGLEWMGGIIPIFGTANYAQKFQGRVTITADKSTSTAYMELSSLRSEDTAVYYCARSPRRAYHDAFDIWGQGTMVTVSSGGGGSGGGGSGGGGSSYELTQPPSMSVAPGKTASITCGGDHIGSKSVHWYQQKPGQAPVLVVYDDSDRPSGIPERFEGSNSGNEAELTISGTQAMDEADYYCLAWDSSTAIFGGGTQLTVLV

SEQ ID NO: 46 - protein, 241 aa, synthetic construct
QLVQSGAEVKKPGSSVKVSCKASGGTFSSYAISWVRQAPGQGLEWMGGIIPIFGTANYAQKFQGRVTITADKSTSTAYMELSSLRSEDTAVYYCARSPRRAYHDAFDIWGQGTMVTVSSGGGGSGGGGSGGGGSSYELTQPPSMSVAPGKTASITCGGDHIGSKSVHWYQQKPGQAPVLVVYDDSDRPSGIPDRFSGSNSGNTATLDIDGTQAMDEADYYCLAWDSSTAIFGGGTQLTVLV

SEQ ID NO: 47 - protein, 7 aa, synthetic construct
GVSLPDY

SEQ ID NO: 48 - protein, 10 aa, synthetic construct
YYYGGSYAMD

SEQ ID NO: 49 - protein, 7 aa, synthetic construct
SQDISKY

SEQ ID NO: 50 - protein, 6 aa, synthetic construct
GNTLPY

SEQ ID NO: 51 - protein, 242 aa, synthetic construct
DIQMTQTTSSLSASLGDRVTISCRASQDISKYLNWYQQKPDGTVKLLIYHTSRLHSGVPSRFSGSGSGTDYSLTISNLEQEDIATYFCQQGNTLPYTFGGGTKLEITGGGGSGGGGSGGGGSEVKLQESGPGLVAPSQSLSVTCTVSGVSLPDYGVSWIRQPPRKGLEWLGVIWGSETTYYNSALKSRLTIIKDNSKSQVFLKMNSLQTDDTAIYYCAKHYYYGGSYAMDYWGQGTSVTVSS

SEQ ID NO: 52 - protein, 242 aa, synthetic construct
DIQMTQTTSSLSASLGDRVTISCRASQDISKYLNWYQQKPDGTVKLLIYHTSRLHSGVPSRFSGSGEGTEYELTISNLEQEDIATYFCQQGNTLPYTFGGGTKLEITGGGGSGGGGSGGGGSEVKLQESGPGLVAPSQSLSVTCTVSGVSLPDYGVSWIRQPPRKGLEWLGVIWGSETTYYNSALKSRLTIIKDNSKSQVFLKMNSLQTDDTAIYYCAKHYYYGGSYAMDYWGQGTSVTVSS

SEQ ID NO: 53 - protein, 242 aa, synthetic construct
DIQMTQTTSSLSASLGDRVTISCRASQDISKYLNWYQQKPDGTVKLLIYHTSRLHSGVPSRFDGDGDGTDYSLTISNLEQEDIATYFCQQGNTLPYTFGGGTKLEITGGGGSGGGGSGGGGSEVKLQESGPGLVAPSQSLSVTCTVSGVSLPDYGVSWIRQPPRKGLEWLGVIWGSETTYYNSALKSRLTIIKDNSKSQVFLKMNSLQTDDTAIYYCAKHYYYGGSYAMDYWGQGTSVTVSS

SEQ ID NO: 54 - protein, 242 aa, synthetic construct
DIQMTQTTSSLSASLGDRVTISCRASQDISKYLNWYQQKPDGTVKLLIYHTSRLHSGVPDRFDGDGSGTDYSLTISNLEQEDIATYFCQQGNTLPYTFGGGTKLEITGGGGSGGGGSGGGGSEVKLQESGPGLVAPSQSLSVTCTVSGVSLPDYGVSWIRQPPRKGLEWLGVIWGSETTYYNSALKSRLTIIKDNSKSQVFLKMNSLQTDDTAIYYCAKHYYYGGSYAMDYWGQGTSVTVSS

SEQ ID NO: 55 - protein, 242 aa, synthetic construct
DIQMTQTTSSLSASLGDRVTISCRASQDISKYLNWYQQKPDGTVKLLIYHTSRLHSGVPSRFSGSGSGTEYELEISNLEQEDIATYFCQQGNTLPYTFGGGTKLEITGGGGSGGGGSGGGGSEVKLQESGPGLVAPSQSLSVTCTVSGVSLPDYGVSWIRQPPRKGLEWLGVIWGSETTYYNSALKSRLTIIKDNSKSQVFLKMNSLQTDDTAIYYCAKHYYYGGSYAMDYWGQGTSVTVSS

SEQ ID NO: 56 - protein, 242 aa, synthetic construct
DIQMTQTTSSLSASLGDRVTISCRASQDISKYLNWYQQKPDGTVKLLIYHTSRLHSGVPSRFDGDGSGTDYDLTISNLEQEDIATYFCQQGNTLPYTFGGGTKLEITGGGGSGGGGSGGGGSEVKLQESGPGLVAPSQSLSVTCTVSGVSLPDYGVSWIRQPPRKGLEWLGVIWGSETTYYNSALKSRLTIIKDNSKSQVFLKMNSLQTDDTAIYYCAKHYYYGGSYAMDYWGQGTSVTVSS

SEQ ID NO: 57 - protein, 242 aa, synthetic construct
DIQMTQTTSSLSASLGDRVTISCRASQDISKYLNWYQQKPDGTVKLLIYHTSRLHSGVPSRFDGSGDGTDYDLTISNLEQEDIATYFCQQGNTLPYTFGGGTKLEITGGGGSGGGGSGGGGSEVKLQESGPGLVAPSQSLSVTCTVSGVSLPDYGVSWIRQPPRKGLEWLGVIWGSETTYYNSALKSRLTIIKDNSKSQVFLKMNSLQTDDTAIYYCAKHYYYGGSYAMDYWGQGTSVTVSS

SEQ ID NO: 58 - protein, 242 aa, synthetic construct
DIQMTQTTSSLSASLGDRVTISCRASQDISKYLNWYQQKPDGTVKLLIYHTSRLHSGVPSRFDGDGDGTDYDLTISNLEQEDIATYFCQQGNTLPYTFGGGTKLEITGGGGSGGGGSGGGGSEVKLQESGPGLVAPSQSLSVTCTVSGVSLPDYGVSWIRQPPRKGLEWLGVIWGSETTYYNSALKSRLTIIKDNSKSQVFLKMNSLQTDDTAIYYCAKHYYYGGSYAMDYWGQGTSVTVSS

SEQ ID NO: 59 - protein, 242 aa, synthetic construct
DIQMTQTTSSLSASLGDRVTISCRASQDISKYLNWYQQKPDGTVKLLIYHTSRLHSGVPSRFEGEGEGTEYELTISNLEQEDIATYFCQQGNTLPYTFGGGTKLEITGGGGSGGGGSGGGGSEVKLQESGPGLVAPSQSLSVTCTVSGVSLPDYGVSWIRQPPRKGLEWLGVIWGSETTYYNSALKSRLTIIKDNSKSQVFLKMNSLQTDDTAIYYCAKHYYYGGSYAMDYWGQGTSVTVSS

SEQ ID NO: 60 - protein, 23 aa, synthetic construct
YIWAPLAGTCGVLLLSLVITLYC

SEQ ID NO: 61 - protein, 28 aa, synthetic construct
FWVLVVVGGVLACYSLLVTVAFIIFWVR

SEQ ID NO: 62 - protein, 106 aa, synthetic construct
GQPKANPTVTLFPPSSEELQANKATLVCLISDFYPGAVTVAWKADGSPVKAGVETTKPSKQSNNKYAASSYLSLTPEQWKSHRSYSCQVTHEGSTVEKTVAPTECS

SEQ ID NO: 63 - protein, 39 aa, synthetic construct
IEVMYPPPYLDNEKSNGTIIHVKGKHLCPSPLFPGPSKP

SEQ ID NO: 64 - protein, 114 aa, synthetic construct
LRVKFSRSADAPAYQQGQNQLYNELNLGRREEYDVLDKRRGRDPEMGGKPQRRKNPQEGLYNELQKDKMAEAYSEIGMKGERRRGKGHDGLYQGLSTATKDTYDALHMQALPPR

SEQ ID NO: 65 - protein, 41 aa, synthetic construct
KRGRKKLLYIFKQPFMRPVQTTQEEDGCSCRFPEEEEGGCE

SEQ ID NO: 66 - protein, 40 aa, synthetic construct
SKRSRLLHSDYMNMTPRRPGPTRKHYQPYAPPRDFAAYRS

SEQ ID NO: 67 - protein, 49 aa, synthetic construct
RSQCMWPRETQLLLEVPPSTEDARSCQFPEEERGERSAEEKGRLGDLWV

SEQ ID NO: 68 - DNA, 24 bp, synthetic construct
  source 1..24: mol_type = other DNA
gatgaggctgactattactgtctg

SEQ ID NO: 69 - DNA, 25 bp, synthetic construct
  source 1..25: mol_type = other DNA
ccggtcgctatcatcatagacgacc

SEQ ID NO: 70 - DNA, 114 bp, synthetic construct
  source 1..114: mol_type = other DNA
gatgatagcgaccggccctcagggatccctgagcgattcgagggcgagaacgaggggaacgaggccactctgaccatcagcgggacccaggctatggatgaggctgactattac

SEQ ID NO: 71 - DNA, 114 bp, synthetic construct
  source 1..114: mol_type = other DNA
gatgatagcgaccggccctcagggatccctgagcgattcgagggcgagaacgaggggaacacagccgagctgaccatcagcgggacccaggctatggatgaggctgactattac

SEQ ID NO: 72 - DNA, 114 bp, synthetic construct
  source 1..114: mol_type = other DNA
gatgatagcgaccggccctcagggatccctgagcgattctctggcgagaacgaggggaacgaggccgagctgaccatcagcgggacccaggctatggatgaggctgactattac

SEQ ID NO: 73 - DNA, 1707 bp, synthetic construct
  source 1..1707: mol_type = other DNA
atgaaacacctgtggttcttcctcctgctggtggcagctcccagatgggtcctgtcccaggtgcagctgcaggtccagctggtacagtctggggctgaggtgaagaagcctgggtcctcggtgaaggtctcctgcaaggcttctggaggcaccttcagcagctatgctatcagctgggtgcgacaggcccctggacaagggcttgagtggatgggagggatcatccctatctttggtacagcaaactacgcacagaagttccagggcagagtcacgattaccgcggacaaatccacgagcacagcctacatggagctgagcagcctgagatctgaggacacggccgtgtattactgtgcgagatccccccggcgggcatatcatgatgcttttgatatctggggccaagggacaatggtcaccgtctcttcaggtggaggcggttcaggcggaggtggcagcggcggtggcgggagttcctatgagctgactcagccaccctcgatgtcagtggccccaggaaagacggccagcattacctgtggcggagaccatattggaagtaaaagtgttcactggtaccagcagaagccaggccaggcccctgtactggtcgtctatgatgatagcgaccggccctcagggatccctgagcgattctctggctccaactctgggaacacagccactctgaccatcagcgggacccaggctatggatgaggctgactattactgtctggcgtgggacagcagcactgcgatcttcggcggaggcacccagctgaccgtcctcgtgggtcagcccaaggccaaccccactgtcactctgtttccgccctcctctgaggagctccaagccaacaaggccacactagtgtgtctgatcagtgacttctacccgggagctgtgacagtggcctggaaggcagatggcagccccgtcaaggcgggagtggagaccaccaaaccctccaaacagagcaacaacaagtacgcggccagcagctacctgagcctgacgcccgagcagtggaagtcccacagaagctacagctgccaggtcacgcatgaagggagcaccgtggagaagactgtggcccctacagaatgttcggcgcgccagactagattttgggtgctggtggtggttggtggagtcctggcttgctatagcttgctagtaacagtggcctttattattttctgggtgaggctgagagtgaagttcagcaggagcgcagacgcccccgcgtaccagcagggccagaaccagctctataacgagctcaatctaggacgaagagaggagtacgatgttttggacaagagacgtggccgggaccctgagatggggggaaagccgcagagaaggaagaaccctcaggaaggcctgtacaatgaactgcagaaagataagatggcggaggcctacagtgagattgggatgaaaggcgagcgccggaggggcaaggggcacgatggcctttaccagggtctcagtacagccaccaaggacacctacgacgcccttcacatgcaggccctgccccctcgcaggagtcagtgcatgtggccccgagagacccagctgctgctggaggtgccgccgtcgaccgaagacgccagaagctgccagttccccgaggaagagcggggcgagcgatcggcagaggagaaggggcggctgggagacctgtgggtgtaa

SEQ ID NO: 74 - DNA, 1707 bp, synthetic construct
  source 1..1707: mol_type = other DNA
atgaaacacctgtggttcttcctcctgctggtggcagctcccagatgggtcctgtcccaggtgcagctgcaggtccagctggtacagtctggggctgaggtgaagaagcctgggtcctcggtgaaggtctcctgcaaggcttctggaggcaccttcagcagctatgctatcagctgggtgcgacaggcccctggacaagggcttgagtggatgggagggatcatccctatctttggtacagcaaactacgcacagaagttccagggcagagtcacgattaccgcggacaaatccacgagcacagcctacatggagctgagcagcctgagatctgaggacacggccgtgtattactgtgcgagatccccccggcgggcatatcatgatgcttttgatatctggggccaagggacaatggtcaccgtctcttcaggtggaggcggttcaggcggaggtggcagcggcggtggcgggagttcctatgagctgactcagccaccctcgatgtcagtggccccaggaaagacggccagcattacctgtggcggagaccatattggaagtaaaagtgttcactggtaccagcagaagccaggccaggcccctgtactggtcgtctatgatgatagcgaccggccctcagggatccctgagcgattcgagggcgagaacgaggggaacgaggccactctgaccatcagcgggacccaggctatggatgaggctgactattactgtctggcgtgggacagcagcactgcgatcttcggcggaggcacccagctgaccgtcctcgtgggtcagcccaaggccaaccccactgtcactctgtttccgccctcctctgaggagctccaagccaacaaggccacactagtgtgtctgatcagtgacttctacccgggagctgtgacagtggcctggaaggcagatggcagccccgtcaaggcgggagtggagaccaccaaaccctccaaacagagcaacaacaagtacgcggccagcagctacctgagcctgacgcccgagcagtggaagtcccacagaagctacagctgccaggtcacgcatgaagggagcaccgtggagaagactgtggcccctacagaatgttcggcgcgccagactagattttgggtgctggtggtggttggtggagtcctggcttgctatagcttgctagtaacagtggcctttattattttctgggtgaggctgagagtgaagttcagcaggagcgcagacgcccccgcgtaccagcagggccagaaccagctctataacgagctcaatctaggacgaagagaggagtacgatgttttggacaagagacgtggccgggaccctgagatggggggaaagccgcagagaaggaagaaccctcaggaaggcctgtacaatgaactgcagaaagataagatggcggaggcctacagtgagattgggatgaaaggcgagcgccggaggggcaaggggcacgatggcctttaccagggtctcagtacagccaccaaggacacctacgacgcccttcacatgcaggccctgccccctcgcaggagtcagtgcatgtggccccgagagacccagctgctgctggaggtgccgccgtcgaccgaagacgccagaagctgccagttccccgaggaagagcggggcgagcgatcggcagaggagaaggggcggctgggagacctgtgggtgtaa

SEQ ID NO: 75 - DNA, 1707 bp, synthetic construct
  source 1..1707: mol_type = other DNA
atgaaacacctgtggttcttcctcctgctggtggcagctcccagatgggtcctgtcccaggtgcagctgcaggtccagctggtacagtctggggctgaggtgaagaagcctgggtcctcggtgaaggtctcctgcaaggcttctggaggcaccttcagcagctatgctatcagctgggtgcgacaggcccctggacaagggcttgagtggatgggagggatcatccctatctttggtacagcaaactacgcacagaagttccagggcagagtcacgattaccgcggacaaatccacgagcacagcctacatggagctgagcagcctgagatctgaggacacggccgtgtattactgtgcgagatccccccggcgggcatatcatgatgcttttgatatctggggccaagggacaatggtcaccgtctcttcaggtggaggcggttcaggcggaggtggcagcggcggtggcgggagttcctatgagctgactcagccaccctcgatgtcagtggccccaggaaagacggccagcattacctgtggcggagaccatattggaagtaaaagtgttcactggtaccagcagaagccaggccaggcccctgtactggtcgtctatgatgatagcgaccggccctcagggatccctgagcgattcgagggcgagaacgaggggaacacagccgagctgaccatcagcgggacccaggctatggatgaggctgactattactgtctggcgtgggacagcagcactgcgatcttcggcggaggcacccagctgaccgtcctcgtgggtcagcccaaggccaaccccactgtcactctgtttccgccctcctctgaggagctccaagccaacaaggccacactagtgtgtctgatcagtgacttctacccgggagctgtgacagtggcctggaaggcagatggcagccccgtcaaggcgggagtggagaccaccaaaccctccaaacagagcaacaacaagtacgcggccagcagctacctgagcctgacgcccgagcagtggaagtcccacagaagctacagctgccaggtcacgcatgaagggagcaccgtggagaagactgtggcccctacagaatgttcggcgcgccagactagattttgggtgctggtggtggttggtggagtcctggcttgctatagcttgctagtaacagtggcctttattattttctgggtgaggctgagagtgaagttcagcaggagcgcagacgcccccgcgtaccagcagggccagaaccagctctataacgagctcaatctaggacgaagagaggagtacgatgttttggacaagagacgtggccgggaccctgagatggggggaaagccgcagagaaggaagaaccctcaggaaggcctgtacaatgaactgcagaaagataagatggcggaggcctacagtgagattgggatgaaaggcgagcgccggaggggcaaggggcacgatggcctttaccagggtctcagtacagccaccaaggacacctacgacgcccttcacatgcaggccctgccccctcgcaggagtcagtgcatgtggccccgagagacccagctgctgctggaggtgccgccgtcgaccgaagacgccagaagctgccagttccccgaggaagagcggggcgagcgatcggcagaggagaaggggcggctgggagacctgtgggtgtaa

SEQ ID NO: 76 - DNA, 1707 bp, synthetic construct
  source 1..1707: mol_type = other DNA
atgaaacacctgtggttcttcctcctgctggtggcagctcccagatgggtcctgtcccaggtgcagctgcaggtccagctggtacagtctggggctgaggtgaagaagcctgggtcctcggtgaaggtctcctgcaaggcttctggaggcaccttcagcagctatgctatcagctgggtgcgacaggcccctggacaagggcttgagtggatgggagggatcatccctatctttggtacagcaaactacgcacagaagttccagggcagagtcacgattaccgcggacaaatccacgagcacagcctacatggagctgagcagcctgagatctgaggacacggccgtgtattactgtgcgagatccccccggcgggcatatcatgatgcttttgatatctggggccaagggacaatggtcaccgtctcttcaggtggaggcggttcaggcggaggtggcagcggcggtggcgggagttcctatgagctgactcagccaccctcgatgtcagtggccccaggaaagacggccagcattacctgtggcggagaccatattggaagtaaaagtgttcactggtaccagcagaagccaggccaggcccctgtactggtcgtctatgatgatagcgaccggccctcagggatccctgagcgattctctggcgagaacgaggggaacgaggccgagctgaccatcagcgggacccaggctatggatgaggctgactattactgtctggcgtgggacagcagcactgcgatcttcggcggaggcacccagctgaccgtcctcgtgggtcagcccaaggccaaccccactgtcactctgtttccgccctcctctgaggagctccaagccaacaaggccacactagtgtgtctgatcagtgacttctacccgggagctgtgacagtggcctggaaggcagatggcagccccgtcaaggcgggagtggagaccaccaaaccctccaaacagagcaacaacaagtacgcggccagcagctacctgagcctgacgcccgagcagtggaagtcccacagaagctacagctgccaggtcacgcatgaagggagcaccgtggagaagactgtggcccctacagaatgttcggcgcgccagactagattttgggtgctggtggtggttggtggagtcctggcttgctatagcttgctagtaacagtggcctttattattttctgggtgaggctgagagtgaagttcagcaggagcgcagacgcccccgcgtaccagcagggccagaaccagctctataacgagctcaatctaggacgaagagaggagtacgatgttttggacaagagacgtggccgggaccctgagatggggggaaagccgcagagaaggaagaaccctcaggaaggcctgtacaatgaactgcagaaagataagatggcggaggcctacagtgagattgggatgaaaggcgagcgccggaggggcaaggggcacgatggcctttaccagggtctcagtacagccaccaaggacacctacgacgcccttcacatgcaggccctgccccctcgcaggagtcagtgcatgtggccccgagagacccagctgctgctggaggtgccgccgtcgaccgaagacgccagaagctgccagttccccgaggaagagcggggcgagcgatcggcagaggagaaggggcggctgggagacctgtgggtgtaa

SEQ ID NO: 77 - protein, 568 aa, synthetic construct
MKHLWFFLLLVAAPRWVLSQVQLQVQLVQSGAEVKKPGSSVKVSCKASGGTFSSYAISWVRQAPGQGLEWMGGIIPIFGTANYAQKFQGRVTITADKSTSTAYMELSSLRSEDTAVYYCARSPRRAYHDAFDIWGQGTMVTVSSGGGGSGGGGSGGGGSSYELTQPPSMSVAPGKTASITCGGDHIGSKSVHWYQQKPGQAPVLVVYDDSDRPSGIPERFSGSNSGNTATLTISGTQAMDEADYYCLAWDSSTAIFGGGTQLTVLVGQPKANPTVTLFPPSSEELQANKATLVCLISDFYPGAVTVAWKADGSPVKAGVETTKPSKQSNNKYAASSYLSLTPEQWKSHRSYSCQVTHEGSTVEKTVAPTECSARQTRFWVLVVVGGVLACYSLLVTVAFIIFWVRLRVKFSRSADAPAYQQGQNQLYNELNLGRREEYDVLDKRRGRDPEMGGKPQRRKNPQEGLYNELQKDKMAEAYSEIGMKGERRRGKGHDGLYQGLSTATKDTYDALHMQALPPRRSQCMWPRETQLLLEVPPSTEDARSCQFPEEERGERSAEEKGRLGDLWV

SEQ ID NO: 78 - protein, 568 aa, synthetic construct
MKHLWFFLLLVAAPRWVLSQVQLQVQLVQSGAEVKKPGSSVKVSCKASGGTFSSYAISWVRQAPGQGLEWMGGIIPIFGTANYAQKFQGRVTITADKSTSTAYMELSSLRSEDTAVYYCARSPRRAYHDAFDIWGQGTMVTVSSGGGGSGGGGSGGGGSSYELTQPPSMSVAPGKTASITCGGDHIGSKSVHWYQQKPGQAPVLVVYDDSDRPSGIPERFEGENEGNEATLTISGTQAMDEADYYCLAWDSSTAIFGGGTQLTVLVGQPKANPTVTLFPPSSEELQANKATLVCLISDFYPGAVTVAWKADGSPVKAGVETTKPSKQSNNKYAASSYLSLTPEQWKSHRSYSCQVTHEGSTVEKTVAPTECSARQTRFWVLVVVGGVLACYSLLVTVAFIIFWVRLRVKFSRSADAPAYQQGQNQLYNELNLGRREEYDVLDKRRGRDPEMGGKPQRRKNPQEGLYNELQKDKMAEAYSEIGMKGERRRGKGHDGLYQGLSTATKDTYDALHMQALPPRRSQCMWPRETQLLLEVPPSTEDARSCQFPEEERGERSAEEKGRLGDLWV

SEQ ID NO: 79 - protein, 568 aa, synthetic construct
MKHLWFFLLLVAAPRWVLSQVQLQVQLVQSGAEVKKPGSSVKVSCKASGGTFSSYAISWVRQAPGQGLEWMGGIIPIFGTANYAQKFQGRVTITADKSTSTAYMELSSLRSEDTAVYYCARSPRRAYHDAFDIWGQGTMVTVSSGGGGSGGGGSGGGGSSYELTQPPSMSVAPGKTASITCGGDHIGSKSVHWYQQKPGQAPVLVVYDDSDRPSGIPERFEGENEGNTAELTISGTQAMDEADYYCLAWDSSTAIFGGGTQLTVLVGQPKANPTVTLFPPSSEELQANKATLVCLISDFYPGAVTVAWKADGSPVKAGVETTKPSKQSNNKYAASSYLSLTPEQWKSHRSYSCQVTHEGSTVEKTVAPTECSARQTRFWVLVVVGGVLACYSLLVTVAFIIFWVRLRVKFSRSADAPAYQQGQNQLYNELNLGRREEYDVLDKRRGRDPEMGGKPQRRKNPQEGLYNELQKDKMAEAYSEIGMKGERRRGKGHDGLYQGLSTATKDTYDALHMQALPPRRSQCMWPRETQLLLEVPPSTEDARSCQFPEEERGERSAEEKGRLGDLWV

SEQ ID NO: 80 - protein, 568 aa, synthetic construct
MKHLWFFLLLVAAPRWVLSQVQLQVQLVQSGAEVKKPGSSVKVSCKASGGTFSSYAISWVRQAPGQGLEWMGGIIPIFGTANYAQKFQGRVTITADKSTSTAYMELSSLRSEDTAVYYCARSPRRAYHDAFDIWGQGTMVTVSSGGGGSGGGGSGGGGSSYELTQPPSMSVAPGKTASITCGGDHIGSKSVHWYQQKPGQAPVLVVYDDSDRPSGIPERFSGENEGNEAELTISGTQAMDEADYYCLAWDSSTAIFGGGTQLTVLVGQPKANPTVTLFPPSSEELQANKATLVCLISDFYPGAVTVAWKADGSPVKAGVETTKPSKQSNNKYAASSYLSLTPEQWKSHRSYSCQVTHEGSTVEKTVAPTECSARQTRFWVLVVVGGVLACYSLLVTVAFIIFWVRLRVKFSRSADAPAYQQGQNQLYNELNLGRREEYDVLDKRRGRDPEMGGKPQRRKNPQEGLYNELQKDKMAEAYSEIGMKGERRRGKGHDGLYQGLSTATKDTYDALHMQALPPRRSQCMWPRETQLLLEVPPSTEDARSCQFPEEERGERSAEEKGRLGDLWV

SEQ ID NO: 81 - DNA, 114 bp, synthetic construct
  source 1..114: mol_type = other DNA
gatgatagcgaccggccatcagggatccctgagcgattcgaaggctccaactctgggaacgaggccgaactgaccatcagcgggacccaggctatggatgaggctgactattac

SEQ ID NO: 82 - DNA, 114 bp, synthetic construct
  source 1..114: mol_type = other DNA
gatgatagcgaccggccatcagggatccctgaccgattctctggctccaactctgggaacacagccactctggacatcgacgggacccaggctatggatgaggctgactattac

SEQ ID NO: 83 - DNA, 1707 bp, synthetic construct
  source 1..1707: mol_type = other DNA
atgaaacacctgtggttcttcctcctgctggtggcagctcccagatgggtcctgtcccaggtgcagctgcaggtccagctggtacagtctggggctgaggtgaagaagcctgggtcctcggtgaaggtctcctgcaaggcttctggaggcaccttcagcagctatgctatcagctgggtgcgacaggcccctggacaagggcttgagtggatgggagggatcatccctatctttggtacagcaaactacgcacagaagttccagggcagagtcacgattaccgcggacaaatccacgagcacagcctacatggagctgagcagcctgagatctgaggacacggccgtgtattactgtgcgagatccccccggcgggcatatcatgatgcttttgatatctggggccaagggacaatggtcaccgtctcttcaggtggaggcggttcaggcggaggtggcagcggcggtggcgggagttcctatgagctgactcagccaccctcgatgtcagtggccccaggaaagacggccagcattacctgtggcggagaccatattggaagtaaaagtgttcactggtaccagcagaagccaggccaggcccctgtactggtcgtctatgatgatagcgaccggccatcagggatccctgagcgattcgaaggctccaactctgggaacgaggccgaactgaccatcagcgggacccaggctatggatgaggctgactattactgtctggcgtgggacagcagcactgcgatcttcggcggaggcacccagctgaccgtcctcgtgggtcagcccaaggccaaccccactgtcactctgtttccgccctcctctgaggagctccaagccaacaaggccacactagtgtgtctgatcagtgacttctacccgggagctgtgacagtggcctggaaggcagatggcagccccgtcaaggcgggagtggagaccaccaaaccctccaaacagagcaacaacaagtacgcggccagcagctacctgagcctgacgcccgagcagtggaagtcccacagaagctacagctgccaggtcacgcatgaagggagcaccgtggagaagactgtggcccctacagaatgttcggcgcgccagactagattttgggtgctggtggtggttggtggagtcctggcttgctatagcttgctagtaacagtggcctttattattttctgggtgaggctgagagtgaagttcagcaggagcgcagacgcccccgcgtaccagcagggccagaaccagctctataacgagctcaatctaggacgaagagaggagtacgatgttttggacaagagacgtggccgggaccctgagatggggggaaagccgcagagaaggaagaaccctcaggaaggcctgtacaatgaactgcagaaagataagatggcggaggcctacagtgagattgggatgaaaggcgagcgccggaggggcaaggggcacgatggcctttaccagggtctcagtacagccaccaaggacacctacgacgcccttcacatgcaggccctgccccctcgcaggagtcagtgcatgtggccccgagagacccagctgctgctggaggtgccgccgtcgaccgaagacgccagaagctgccagttccccgaggaagagcggggcgagcgatcggcagaggagaaggggcggctgggagacctgtgggtgtaa

SEQ ID NO: 84 - DNA, 1707 bp, synthetic construct
  source 1..1707: mol_type = other DNA
atgaaacacctgtggttcttcctcctgctggtggcagctcccagatgggtcctgtcccaggtgcagctgcaggtccagctggtacagtctggggctgaggtgaagaagcctgggtcctcggtgaaggtctcctgcaaggcttctggaggcaccttcagcagctatgctatcagctgggtgcgacaggcccctggacaagggcttgagtggatgggagggatcatccctatctttggtacagcaaactacgcacagaagttccagggcagagtcacgattaccgcggacaaatccacgagcacagcctacatggagctgagcagcctgagatctgaggacacggccgtgtattactgtgcgagatccccccggcgggcatatcatgatgcttttgatatctggggccaagggacaatggtcaccgtctcttcaggtggaggcggttcaggcggaggtggcagcggcggtggcgggagttcctatgagctgactcagccaccctcgatgtcagtggccccaggaaagacggccagcattacctgtggcggagaccatattggaagtaaaagtgttcactggtaccagcagaagccaggccaggcccctgtactggtcgtctatgatgatagcgaccggccatcagggatccctgaccgattctctggctccaactctgggaacacagccactctggacatcgacgggacccaggctatggatgaggctgactattactgtctggcgtgggacagcagcactgcgatcttcggcggaggcacccagctgaccgtcctcgtgggtcagcccaaggccaaccccactgtcactctgtttccgccctcctctgaggagctccaagccaacaaggccacactagtgtgtctgatcagtgacttctacccgggagctgtgacagtggcctggaaggcagatggcagccccgtcaaggcgggagtggagaccaccaaaccctccaaacagagcaacaacaagtacgcggccagcagctacctgagcctgacgcccgagcagtggaagtcccacagaagctacagctgccaggtcacgcatgaagggagcaccgtggagaagactgtggcccctacagaatgttcggcgcgccagactagattttgggtgctggtggtggttggtggagtcctggcttgctatagcttgctagtaacagtggcctttattattttctgggtgaggctgagagtgaagttcagcaggagcgcagacgcccccgcgtaccagcagggccagaaccagctctataacgagctcaatctaggacgaagagaggagtacgatgttttggacaagagacgtggccgggaccctgagatggggggaaagccgcagagaaggaagaaccctcaggaaggcctgtacaatgaactgcagaaagataagatggcggaggcctacagtgagattgggatgaaaggcgagcgccggaggggcaaggggcacgatggcctttaccagggtctcagtacagccaccaaggacacctacgacgcccttcacatgcaggccctgccccctcgcaggagtcagtgcatgtggccccgagagacccagctgctgctggaggtgccgccgtcgaccgaagacgccagaagctgccagttccccgaggaagagcggggcgagcgatcggcagaggagaaggggcggctgggagacctgtgggtgtaa

SEQ ID NO: 85 - protein, 568 aa, synthetic construct
MKHLWFFLLLVAAPRWVLSQVQLQVQLVQSGAEVKKPGSSVKVSCKASGGTFSSYAISWVRQAPGQGLEWMGGIIPIFGTANYAQKFQGRVTITADKSTSTAYMELSSLRSEDTAVYYCARSPRRAYHDAFDIWGQGTMVTVSSGGGGSGGGGSGGGGSSYELTQPPSMSVAPGKTASITCGGDHIGSKSVHWYQQKPGQAPVLVVYDDSDRPSGIPERFEGSNSGNEAELTISGTQAMDEADYYCLAWDSSTAIFGGGTQLTVLVGQPKANPTVTLFPPSSEELQANKATLVCLISDFYPGAVTVAWKADGSPVKAGVETTKPSKQSNNKYAASSYLSLTPEQWKSHRSYSCQVTHEGSTVEKTVAPTECSARQTRFWVLVVVGGVLACYSLLVTVAFIIFWVRLRVKFSRSADAPAYQQGQNQLYNELNLGRREEYDVLDKRRGRDPEMGGKPQRRKNPQEGLYNELQKDKMAEAYSEIGMKGERRRGKGHDGLYQGLSTATKDTYDALHMQALPPRRSQCMWPRETQLLLEVPPSTEDARSCQFPEEERGERSAEEKGRLGDLWV

SEQ ID NO: 86 - protein, 568 aa, synthetic construct
MKHLWFFLLLVAAPRWVLSQVQLQVQLVQSGAEVKKPGSSVKVSCKASGGTFSSYAISWVRQAPGQGLEWMGGIIPIFGTANYAQKFQGRVTITADKSTSTAYMELSSLRSEDTAVYYCARSPRRAYHDAFDIWGQGTMVTVSSGGGGSGGGGSGGGGSSYELTQPPSMSVAPGKTASITCGGDHIGSKSVHWYQQKPGQAPVLVVYDDSDRPSGIPDRFSGSNSGNTATLDIDGTQAMDEADYYCLAWDSSTAIFGGGTQLTVLVGQPKANPTVTLFPPSSEELQANKATLVCLISDFYPGAVTVAWKADGSPVKAGVETTKPSKQSNNKYAASSYLSLTPEQWKSHRSYSCQVTHEGSTVEKTVAPTECSARQTRFWVLVVVGGVLACYSLLVTVAFIIFWVRLRVKFSRSADAPAYQQGQNQLYNELNLGRREEYDVLDKRRGRDPEMGGKPQRRKNPQEGLYNELQKDKMAEAYSEIGMKGERRRGKGHDGLYQGLSTATKDTYDALHMQALPPRRSQCMWPRETQLLLEVPPSTEDARSCQFPEEERGERSAEEKGRLGDLWV

SEQ ID NO: 87 - DNA, 24 bp, synthetic construct
  source 1..24: mol_type = other DNA
gatatagccacctatttctgccag

SEQ ID NO: 88 - DNA, 24 bp, synthetic construct
  source 1..24: mol_type = other DNA
tccactatgcagccgagatgtgtg

SEQ ID NO: 89 - DNA, 102 bp, synthetic construct
  source 1..102: mol_type = other DNA
cggctgcatagtggagttccttctcgattttcaggctctggcgaagggacagagtatgaactgacaatctccaacttggaacaggaggatatagccacctat

SEQ ID NO: 90 - DNA, 102 bp, synthetic construct
  source 1..102: mol_type = other DNA
cggctgcatagtggagttccttctcgatttgatggcgatggcgatgggacagattatagtctgacaatctccaacttggaacaggaggatatagccacctat

SEQ ID NO: 91 - protein, 1455 aa, synthetic construct
ATGAAACACCTGTGGTTCTTCCTCCTGCTGGTGGCAGCTCCCAGATGGGTCCTGTCCGACATCCAAATGACGCAGACTACAAGCAGCTTGTCAGCCTCACTGGGAGATCGAGTCACCATTAGCTGCAGAGCTAGCCAGGATATAAGCAAATACCTGAACTGGTATCAGCAGAAACCCGATGGCACCGTGAAGCTGCTGATCTATCACACATCTCGGCTGCATAGTGGAGTTCCTTCTCGATTTTCAGGCTCTGGCTCTGGGACAGATTATAGTCTGACAATCTCCAACTTGGAACAGGAGGATATAGCCACCTATTTCTGCCAGCAAGGGAATACCCTCCCGTATACATTTGGAGGCGGCACTAAGCTGGAGATTACGGGTGGAGGCGGTTCAGGCGGAGGTGGCAGCGGCGGTGGCGGGAGTGAAGTGAAACTGCAGGAGTCAGGCCCAGGCCTTGTCGCACCCTCCCAATCCCTGAGTGTCACATGCACAGTAAGCGGGGTTTCCCTCCCCGACTACGGTGTTTCATGGATCAGACAGCCTCCAAGGAAAGGACTTGAGTGGCTCGGGGTGATTTGGGGTAGCGAAACCACCTACTACAATAGCGCGTTGAAGTCCAGGCTCACCATCATCAAGGATAACAGTAAATCCCAGGTTTTCCTGAAAATGAATAGCCTGCAGACAGATGATACTGCCATATACTACTGCGCCAAACACTATTACTACGGCGGATCTTATGCGATGGACTATTGGGGTCAAGGTACATCTGTAACCGTGAGTTCCACCACCACTCCTGCACCTAGGCCACCCACGCCTGCCCCAACTATTGCATCCCAGCCTCTGTCTCTGCGCCCCGAAGCCTGTCGGCCTGCAGCTGGAGGCGCCGTGCACACTCGGGGCCTCGACTTCGCATGTGATATCTACATTTGGGCTCCACTGGCCGGTACGTGTGGGGTCCTTCTGCTCAGTCTGGTGATCACTCTGTATTGCAAAAGAGGTCGTAAGAAGCTTTTGTACATTTTCAAGCAGCCCTTTATGCGGCCGGTGCAAACAACTCAGGAGGAGGATGGATGTAGCTGTCGGTTTCCAGAGGAAGAGGAGGGAGGTTGCGAACTGCGCGTGAAGTTCTCCAGGAGCGCTGACGCGCCCGCTTACAAGCAGGGGCAGAATCAGCTGTACAACGAATTGAACCTCGGGCGTCGCGAGGAGTATGACGTCCTCGACAAGCGAAGGGGCCGGGACCCGGAAATGGGAGGCAAGCCACGCAGGAAGAATCCCCAAGAGGGACTGTATAACGAGCTCCAGAAGGACAAAATGGCTGAAGCCTACAGCGAAATTGGTATGAAAGGGGAGCGCAGAAGAGGAAAGGGGCATGACGGGCTCTACCAGGGATTGAGCACTGCCACCAAAGACACCTATGACGCTCTGCACATGCAAGCTCTGCCACCTAGATGA

SEQ ID NO: 92 - DNA, 1455 bp, synthetic construct
  source 1..1455: mol_type = other DNA
atgaaacacctgtggttcttcctcctgctggtggcagctcccagatgggtcctgtccgacatccaaatgacgcagactacaagcagcttgtcagcctcactgggagatcgagtcaccattagctgcagagctagccaggatataagcaaatacctgaactggtatcagcagaaacccgatggcaccgtgaagctgctgatctatcacacatctcggctgcatagtggagttccttctcgattttcaggctctggcgaagggacagagtatgaactgacaatctccaacttggaacaggaggatatagccacctatttctgccagcaagggaataccctcccgtatacatttggaggcggcactaagctggagattacgggtggaggcggttcaggcggaggtggcagcggcggtggcgggagtgaagtgaaactgcaggagtcaggcccaggccttgtcgcaccctcccaatccctgagtgtcacatgcacagtaagcggggtttccctccccgactacggtgtttcatggatcagacagcctccaaggaaaggacttgagtggctcggggtgatttggggtagcgaaaccacctactacaatagcgcgttgaagtccaggctcaccatcatcaaggataacagtaaatcccaggttttcctgaaaatgaatagcctgcagacagatgatactgccatatactactgcgccaaacactattactacggcggatcttatgcgatggactattggggtcaaggtacatctgtaaccgtgagttccaccaccactcctgcacctaggccacccacgcctgccccaactattgcatcccagcctctgtctctgcgccccgaagcctgtcggcctgcagctggaggcgccgtgcacactcggggcctcgacttcgcatgtgatatctacatttgggctccactggccggtacgtgtggggtccttctgctcagtctggtgatcactctgtattgcaaaagaggtcgtaagaagcttttgtacattttcaagcagccctttatgcggccggtgcaaacaactcaggaggaggatggatgtagctgtcggtttccagaggaagaggagggaggttgcgaactgcgcgtgaagttctccaggagcgctgacgcgcccgcttacaagcaggggcagaatcagctgtacaacgaattgaacctcgggcgtcgcgaggagtatgacgtcctcgacaagcgaaggggccgggacccggaaatgggaggcaagccacgcaggaagaatccccaagagggactgtataacgagctccagaaggacaaaatggctgaagcctacagcgaaattggtatgaaaggggagcgcagaagaggaaaggggcatgacgggctctaccagggattgagcactgccaccaaagacacctatgacgctctgcacatgcaagctctgccacctagatga

SEQ ID NO: 93 - DNA, 1455 bp, synthetic construct
  source 1..1455: mol_type = other DNA
atgaaacacctgtggttcttcctcctgctggtggcagctcccagatgggtcctgtccgacatccaaatgacgcagactacaagcagcttgtcagcctcactgggagatcgagtcaccattagctgcagagctagccaggatataagcaaatacctgaactggtatcagcagaaacccgatggcaccgtgaagctgctgatctatcacacatctcggctgcatagtggagttccttctcgatttgatggcgatggcgatgggacagattatagtctgacaatctccaacttggaacaggaggatatagccacctatttctgccagcaagggaataccctcccgtatacatttggaggcggcactaagctggagattacgggtggaggcggttcaggcggaggtggcagcggcggtggcgggagtgaagtgaaactgcaggagtcaggcccaggccttgtcgcaccctcccaatccctgagtgtcacatgcacagtaagcggggtttccctccccgactacggtgtttcatggatcagacagcctccaaggaaaggacttgagtggctcggggtgatttggggtagcgaaaccacctactacaatagcgcgttgaagtccaggctcaccatcatcaaggataacagtaaatcccaggttttcctgaaaatgaatagcctgcagacagatgatactgccatatactactgcgccaaacactattactacggcggatcttatgcgatggactattggggtcaaggtacatctgtaaccgtgagttccaccaccactcctgcacctaggccacccacgcctgccccaactattgcatcccagcctctgtctctgcgccccgaagcctgtcggcctgcagctggaggcgccgtgcacactcggggcctcgacttcgcatgtgatatctacatttgggctccactggccggtacgtgtggggtccttctgctcagtctggtgatcactctgtattgcaaaagaggtcgtaagaagcttttgtacattttcaagcagccctttatgcggccggtgcaaacaactcaggaggaggatggatgtagctgtcggtttccagaggaagaggagggaggttgcgaactgcgcgtgaagttctccaggagcgctgacgcgcccgcttacaagcaggggcagaatcagctgtacaacgaattgaacctcgggcgtcgcgaggagtatgacgtcctcgacaagcgaaggggccgggacccggaaatgggaggcaagccacgcaggaagaatccccaagagggactgtataacgagctccagaaggacaaaatggctgaagcctacagcgaaattggtatgaaaggggagcgcagaagaggaaaggggcatgacgggctctaccagggattgagcactgccaccaaagacacctatgacgctctgcacatgcaagctctgccacctagatga

SEQ ID NO: 94 - protein, 484 aa, synthetic construct
MKHLWFFLLLVAAPRWVLSDIQMTQTTSSLSASLGDRVTISCRASQDISKYLNWYQQKPDGTVKLLIYHTSRLHSGVPSRFSGSGSGTDYSLTISNLEQEDIATYFCQQGNTLPYTFGGGTKLEITGGGGSGGGGSGGGGSEVKLQESGPGLVAPSQSLSVTCTVSGVSLPDYGVSWIRQPPRKGLEWLGVIWGSETTYYNSALKSRLTIIKDNSKSQVFLKMNSLQTDDTAIYYCAKHYYYGGSYAMDYWGQGTSVTVSSTTTPAPRPPTPAPTIASQPLSLRPEACRPAAGGAVHTRGLDFACDIYIWAPLAGTCGVLLLSLVITLYCKRGRKKLLYIFKQPFMRPVQTTQEEDGCSCRFPEEEEGGCELRVKFSRSADAPAYKQGQNQLYNELNLGRREEYDVLDKRRGRDPEMGGKPRRKNPQEGLYNELQKDKMAEAYSEIGMKGERRRGKGHDGLYQGLSTATKDTYDALHMQALPPR

SEQ ID NO: 95 - protein, 484 aa, synthetic construct
MKHLWFFLLLVAAPRWVLSDIQMTQTTSSLSASLGDRVTISCRASQDISKYLNWYQQKPDGTVKLLIYHTSRLHSGVPSRFSGSGEGTEYELTISNLEQEDIATYFCQQGNTLPYTFGGGTKLEITGGGGSGGGGSGGGGSEVKLQESGPGLVAPSQSLSVTCTVSGVSLPDYGVSWIRQPPRKGLEWLGVIWGSETTYYNSALKSRLTIIKDNSKSQVFLKMNSLQTDDTAIYYCAKHYYYGGSYAMDYWGQGTSVTVSSTTTPAPRPPTPAPTIASQPLSLRPEACRPAAGGAVHTRGLDFACDIYIWAPLAGTCGVLLLSLVITLYCKRGRKKLLYIFKQPFMRPVQTTQEEDGCSCRFPEEEEGGCELRVKFSRSADAPAYKQGQNQLYNELNLGRREEYDVLDKRRGRDPEMGGKPRRKNPQEGLYNELQKDKMAEAYSEIGMKGERRRGKGHDGLYQGLSTATKDTYDALHMQALPPR

SEQ ID NO: 96 - protein, 484 aa, synthetic construct
MKHLWFFLLLVAAPRWVLSDIQMTQTTSSLSASLGDRVTISCRASQDISKYLNWYQQKPDGTVKLLIYHTSRLHSGVPSRFDGDGDGTDYSLTISNLEQEDIATYFCQQGNTLPYTFGGGTKLEITGGGGSGGGGSGGGGSEVKLQESGPGLVAPSQSLSVTCTVSGVSLPDYGVSWIRQPPRKGLEWLGVIWGSETTYYNSALKSRLTIIKDNSKSQVFLKMNSLQTDDTAIYYCAKHYYYGGSYAMDYWGQGTSVTVSSTTTPAPRPPTPAPTIASQPLSLRPEACRPAAGGAVHTRGLDFACDIYIWAPLAGTCGVLLLSLVITLYCKRGRKKLLYIFKQPFMRPVQTTQEEDGCSCRFPEEEEGGCELRVKFSRSADAPAYKQGQNQLYNELNLGRREEYDVLDKRRGRDPEMGGKPRRKNPQEGLYNELQKDKMAEAYSEIGMKGERRRGKGHDGLYQGLSTATKDTYDALHMQALPPR

SEQ ID NO: 97 - DNA, 102 bp, synthetic construct
  source 1..102: mol_type = other DNA
cggctgcatagtggagttcctgaccgatttgatggcgatggctctgggacagattatagtctgacaatctccaacttggaacaggaggatatagccacctat

SEQ ID NO: 98 - DNA, 102 bp, synthetic construct
  source 1..102: mol_type = other DNA
cggctgcatagtggagttccttctcgattttcaggctctggctctgggacagagtatgaactggagatctccaacttggaacaggaggatatagccacctat

SEQ ID NO: 99 - DNA, 102 bp, synthetic construct
  source 1..102: mol_type = other DNA
cggctgcatagtggagttccttctcgatttgatggcgatggctctgggacagattatgatctgacaatctccaacttggaacaggaggatatagccacctat

SEQ ID NO: 100 - DNA, 102 bp, synthetic construct
  source 1..102: mol_type = other DNA
cggctgcatagtggagttccttctcgatttgatggctctggcgatgggacagattatgatctgacaatctccaacttggaacaggaggatatagccacctat

SEQ ID NO: 101 - DNA, 102 bp, synthetic construct
  source 1..102: mol_type = other DNA
cggctgcatagtggagttccttctcgatttgatggcgatggcgatgggacagattatgatctgacaatctccaacttggaacaggaggatatagccacctat

SEQ ID NO: 102 - DNA, 102 bp, synthetic construct
  source 1..102: mol_type = other DNA
cggctgcatagtggagttccttctcgatttgaaggcgaaggcgaagggacagaatatgaactgacaatctccaacttggaacaggaggatatagccacctat

SEQ ID NO: 103 - DNA, 1449 bp, synthetic construct
  source 1..1449: mol_type = other DNA
atgaaacacctgtggttcttcctcctgctggtggcagctcccagatgggtcctgtccgacatccaaatgacgcagactacaagcagcttgtcagcctcactgggagatcgagtcaccattagctgcagagctagccaggatataagcaaatacctgaactggtatcagcagaaacccgatggcaccgtgaagctgctgatctatcacacatctcggctgcatagtggagttccttctcgattttcaggctctggctctgggacagattatagtctgacaatctccaacttggaacaggaggatatagccacctatttctgccagcaagggaataccctcccgtatacatttggaggcggcactaagctggagattacgggtggaggcggttcaggcggaggtggcagcggcggtggcgggagtgaagtgaaactgcaggagtcaggcccaggccttgtcgcaccctcccaatccctgagtgtcacatgcacagtaagcggggtttccctccccgactacggtgtttcatggatcagacagcctccaaggaaaggacttgagtggctcggggtgatttggggtagcgaaaccacctactacaatagcgcgttgaagtccaggctcaccatcatcaaggataacagtaaatcccaggttttcctgaaaatgaatagcctgcagacagatgatactgccatatactactgcgccaaacactattactacggcggatcttatgcgatggactattggggtcaaggtacatctgtaaccgtgagttccatcgaagtgatgtaccctcctccttacctggacaacgagaagtccaacggcaccatcatccacgtgaagggcaagcacctgtgtccttctccactgttccccggacctagcaagcctttttgggtgctggtggtggttggtggagtcctggcttgctatagcttgctagtaacagtggcctttattattttctgggtgaggagtaagaggagcaggctcctgcacagtgactacatgaacatgactccccgccgccccgggcccacccgcaagcattaccagccctatgccccaccacgcgacttcgcagcctatcgctccctgagagtgaagttcagcaggagcgcagacgcccccgcgtaccagcagggccagaaccagctctataacgagctcaatctaggacgaagagaggagtacgatgttttggacaagagacgtggccgggaccctgagatggggggaaagccgcagagaaggaagaaccctcaggaaggcctgtacaatgaactgcagaaagataagatggcggaggcctacagtgagattgggatgaaaggcgagcgccggaggggcaaggggcacgatggcctttaccagggtctcagtacagccaccaaggacacctacgacgcccttcacatgcaggccctgccccctcgctaa

SEQ ID NO: 104 - DNA, 1449 bp, synthetic construct
  source 1..1449: mol_type = other DNA
atgaaacacctgtggttcttcctcctgctggtggcagctcccagatgggtcctgtccgacatccaaatgacgcagactacaagcagcttgtcagcctcactgggagatcgagtcaccattagctgcagagctagccaggatataagcaaatacctgaactggtatcagcagaaacccgatggcaccgtgaagctgctgatctatcacacatctcggctgcatagtggagttcctgaccgatttgatggcgatggctctgggacagattatagtctgacaatctccaacttggaacaggaggatatagccacctatttctgccagcaagggaataccctcccgtatacatttggaggcggcactaagctggagattacgggtggaggcggttcaggcggaggtggcagcggcggtggcgggagtgaagtgaaactgcaggagtcaggcccaggccttgtcgcaccctcccaatccctgagtgtcacatgcacagtaagcggggtttccctccccgactacggtgtttcatggatcagacagcctccaaggaaaggacttgagtggctcggggtgatttggggtagcgaaaccacctactacaatagcgcgttgaagtccaggctcaccatcatcaaggataacagtaaatcccaggttttcctgaaaatgaatagcctgcagacagatgatactgccatatactactgcgccaaacactattactacggcggatcttatgcgatggactattggggtcaaggtacatctgtaaccgtgagttccatcgaagtgatgtaccctcctccttacctggacaacgagaagtccaacggcaccatcatccacgtgaagggcaagcacctgtgtccttctccactgttccccggacctagcaagcctttttgggtgctggtggtggttggtggagtcctggcttgctatagcttgctagtaacagtggcctttattattttctgggtgaggagtaagaggagcaggctcctgcacagtgactacatgaacatgactccccgccgccccgggcccacccgcaagcattaccagccctatgccccaccacgcgacttcgcagcctatcgctccctgagagtgaagttcagcaggagcgcagacgcccccgcgtaccagcagggccagaaccagctctataacgagctcaatctaggacgaagagaggagtacgatgttttggacaagagacgtggccgggaccctgagatggggggaaagccgcagagaaggaagaaccctcaggaaggcctgtacaatgaactgcagaaagataagatggcggaggcctacagtgagattgggatgaaaggcgagcgccggaggggcaaggggcacgatggcctttaccagggtctcagtacagccaccaaggacacctacgacgcccttcacatgcaggccctgccccctcgctaa

SEQ ID NO: 105 - DNA, 1449 bp, synthetic construct
  source 1..1449: mol_type = other DNA
atgaaacacctgtggttcttcctcctgctggtggcagctcccagatgggtcctgtccgacatccaaatgacgcagactacaagcagcttgtcagcctcactgggagatcgagtcaccattagctgcagagctagccaggatataagcaaatacctgaactggtatcagcagaaacccgatggcaccgtgaagctgctgatctatcacacatctcggctgcatagtggagttccttctcgattttcaggctctggctctgggacagagtatgaactggagatctccaacttggaacaggaggatatagccacctatttctgccagcaagggaataccctcccgtatacatttggaggcggcactaagctggagattacgggtggaggcggttcaggcggaggtggcagcggcggtggcgggagtgaagtgaaactgcaggagtcaggcccaggccttgtcgcaccctcccaatccctgagtgtcacatgcacagtaagcggggtttccctccccgactacggtgtttcatggatcagacagcctccaaggaaaggacttgagtggctcggggtgatttggggtagcgaaaccacctactacaatagcgcgttgaagtccaggctcaccatcatcaaggataacagtaaatcccaggttttcctgaaaatgaatagcctgcagacagatgatactgccatatactactgcgccaaacactattactacggcggatcttatgcgatggactattggggtcaaggtacatctgtaaccgtgagttccatcgaagtgatgtaccctcctccttacctggacaacgagaagtccaacggcaccatcatccacgtgaagggcaagcacctgtgtccttctccactgttccccggacctagcaagcctttttgggtgctggtggtggttggtggagtcctggcttgctatagcttgctagtaacagtggcctttattattttctgggtgaggagtaagaggagcaggctcctgcacagtgactacatgaacatgactccccgccgccccgggcccacccgcaagcattaccagccctatgccccaccacgcgacttcgcagcctatcgctccctgagagtgaagttcagcaggagcgcagacgcccccgcgtaccagcagggccagaaccagctctataacgagctcaatctaggacgaagagaggagtacgatgttttggacaagagacgtggccgggaccctgagatggggggaaagccgcagagaaggaagaaccctcaggaaggcctgtacaatgaactgcagaaagataagatggcggaggcctacagtgagattgggatgaaaggcgagcgccggaggggcaaggggcacgatggcctttaccagggtctcagtacagccaccaaggacacctacgacgcccttcacatgcaggccctgccccctcgctaa

SEQ ID NO: 106 - DNA, 1449 bp, synthetic construct
  source 1..1449: mol_type = other DNA
atgaaacacctgtggttcttcctcctgctggtggcagctcccagatgggtcctgtccgacatccaaatgacgcagactacaagcagcttgtcagcctcactgggagatcgagtcaccattagctgcagagctagccaggatataagcaaatacctgaactggtatcagcagaaacccgatggcaccgtgaagctgctgatctatcacacatctcggctgcatagtggagttccttctcgatttgatggcgatggctctgggacagattatgatctgacaatctccaacttggaacaggaggatatagccacctatttctgccagcaagggaataccctcccgtatacatttggaggcggcactaagctggagattacgggtggaggcggttcaggcggaggtggcagcggcggtggcgggagtgaagtgaaactgcaggagtcaggcccaggccttgtcgcaccctcccaatccctgagtgtcacatgcacagtaagcggggtttccctccccgactacggtgtttcatggatcagacagcctccaaggaaaggacttgagtggctcggggtgatttggggtagcgaaaccacctactacaatagcgcgttgaagtccaggctcaccatcatcaaggataacagtaaatcccaggttttcctgaaaatgaatagcctgcagacagatgatactgccatatactactgcgccaaacactattactacggcggatcttatgcgatggactattggggtcaaggtacatctgtaaccgtgagttccatcgaagtgatgtaccctcctccttacctggacaacgagaagtccaacggcaccatcatccacgtgaagggcaagcacctgtgtccttctccactgttccccggacctagcaagcctttttgggtgctggtggtggttggtggagtcctggcttgctatagcttgctagtaacagtggcctttattattttctgggtgaggagtaagaggagcaggctcctgcacagtgactacatgaacatgactccccgccgccccgggcccacccgcaagcattaccagccctatgccccaccacgcgacttcgcagcctatcgctccctgagagtgaagttcagcaggagcgcagacgcccccgcgtaccagcagggccagaaccagctctataacgagctcaatctaggacgaagagaggagtacgatgttttggacaagagacgtggccgggaccctgagatggggggaaagccgcagagaaggaagaaccctcaggaaggcctgtacaatgaactgcagaaagataagatggcggaggcctacagtgagattgggatgaaaggcgagcgccggaggggcaaggggcacgatggcctttaccagggtctcagtacagccaccaaggacacctacgacgcccttcacatgcaggccctgccccctcgctaa

SEQ ID NO: 107 - DNA, 1449 bp, synthetic construct
  source 1..1449: mol_type = other DNA
atgaaacacctgtggttcttcctcctgctggtggcagctcccagatgggtcctgtccgacatccaaatgacgcagactacaagcagcttgtcagcctcactgggagatcgagtcaccattagctgcagagctagccaggatataagcaaatacctgaactggtatcagcagaaacccgatggcaccgtgaagctgctgatctatcacacatctcggctgcatagtggagttccttctcgatttgatggctctggcgatgggacagattatgatctgacaatctccaacttggaacaggaggatatagccacctatttctgccagcaagggaataccctcccgtatacatttggaggcggcactaagctggagattacgggtggaggcggttcaggcggaggtggcagcggcggtggcgggagtgaagtgaaactgcaggagtcaggcccaggccttgtcgcaccctcccaatccctgagtgtcacatgcacagtaagcggggtttccctccccgactacggtgtttcatggatcagacagcctccaaggaaaggacttgagtggctcggggtgatttggggtagcgaaaccacctactacaatagcgcgttgaagtccaggctcaccatcatcaaggataacagtaaatcccaggttttcctgaaaatgaatagcctgcagacagatgatactgccatatactactgcgccaaacactattactacggcggatcttatgcgatggactattggggtcaaggtacatctgtaaccgtgagttccatcgaagtgatgtaccctcctccttacctggacaacgagaagtccaacggcaccatcatccacgtgaagggcaagcacctgtgtccttctccactgttccccggacctagcaagcctttttgggtgctggtggtggttggtggagtcctggcttgctatagcttgctagtaacagtggcctttattattttctgggtgaggagtaagaggagcaggctcctgcacagtgactacatgaacatgactccccgccgccccgggcccacccgcaagcattaccagccctatgccccaccacgcgacttcgcagcctatcgctccctgagagtgaagttcagcaggagcgcagacgcccccgcgtaccagcagggccagaaccagctctataacgagctcaatctaggacgaagagaggagtacgatgttttggacaagagacgtggccgggaccctgagatggggggaaagccgcagagaaggaagaaccctcaggaaggcctgtacaatgaactgcagaaagataagatggcggaggcctacagtgagattgggatgaaaggcgagcgccggaggggcaaggggcacgatggcctttaccagggtctcagtacagccaccaaggacacctacgacgcccttcacatgcaggccctgccccctcgctaa

SEQ ID NO: 108 - DNA, 1449 bp, synthetic construct
  source 1..1449: mol_type = other DNA
atgaaacacctgtggttcttcctcctgctggtggcagctcccagatgggtcctgtccgacatccaaatgacgcagactacaagcagcttgtcagcctcactgggagatcgagtcaccattagctgcagagctagccaggatataagcaaatacctgaactggtatcagcagaaacccgatggcaccgtgaagctgctgatctatcacacatctcggctgcatagtggagttccttctcgatttgatggcgatggcgatgggacagattatgatctgacaatctccaacttggaacaggaggatatagccacctatttctgccagcaagggaataccctcccgtatacatttggaggcggcactaagctggagattacgggtggaggcggttcaggcggaggtggcagcggcggtggcgggagtgaagtgaaactgcaggagtcaggcccaggccttgtcgcaccctcccaatccctgagtgtcacatgcacagtaagcggggtttccctccccgactacggtgtttcatggatcagacagcctccaaggaaaggacttgagtggctcggggtgatttggggtagcgaaaccacctactacaatagcgcgttgaagtccaggctcaccatcatcaaggataacagtaaatcccaggttttcctgaaaatgaatagcctgcagacagatgatactgccatatactactgcgccaaacactattactacggcggatcttatgcgatggactattggggtcaaggtacatctgtaaccgtgagttccatcgaagtgatgtaccctcctccttacctggacaacgagaagtccaacggcaccatcatccacgtgaagggcaagcacctgtgtccttctccactgttccccggacctagcaagcctttttgggtgctggtggtggttggtggagtcctggcttgctatagcttgctagtaacagtggcctttattattttctgggtgaggagtaagaggagcaggctcctgcacagtgactacatgaacatgactccccgccgccccgggcccacccgcaagcattaccagccctatgccccaccacgcgacttcgcagcctatcgctccctgagagtgaagttcagcaggagcgcagacgcccccgcgtaccagcagggccagaaccagctctataacgagctcaatctaggacgaagagaggagtacgatgttttggacaagagacgtggccgggaccctgagatggggggaaagccgcagagaaggaagaaccctcaggaaggcctgtacaatgaactgcagaaagataagatggcggaggcctacagtgagattgggatgaaaggcgagcgccggaggggcaaggggcacgatggcctttaccagggtctcagtacagccaccaaggacacctacgacgcccttcacatgcaggccctgccccctcgctaa

SEQ ID NO: 109 - DNA, 1449 bp, synthetic construct
  source 1..1449: mol_type = other DNA
atgaaacacctgtggttcttcctcctgctggtggcagctcccagatgggtcctgtccgacatccaaatgacgcagactacaagcagcttgtcagcctcactgggagatcgagtcaccattagctgcagagctagccaggatataagcaaatacctgaactggtatcagcagaaacccgatggcaccgtgaagctgctgatctatcacacatctcggctgcatagtggagttccttctcgatttgaaggcgaaggcgaagggacagaatatgaactgacaatctccaacttggaacaggaggatatagccacctatttctgccagcaagggaataccctcccgtatacatttggaggcggcactaagctggagattacgggtggaggcggttcaggcggaggtggcagcggcggtggcgggagtgaagtgaaactgcaggagtcaggcccaggccttgtcgcaccctcccaatccctgagtgtcacatgcacagtaagcggggtttccctccccgactacggtgtttcatggatcagacagcctccaaggaaaggacttgagtggctcggggtgatttggggtagcgaaaccacctactacaatagcgcgttgaagtccaggctcaccatcatcaaggataacagtaaatcccaggttttcctgaaaatgaatagcctgcagacagatgatactgccatatactactgcgccaaacactattactacggcggatcttatgcgatggactattggggtcaaggtacatctgtaaccgtgagttccatcgaagtgatgtaccctcctccttacctggacaacgagaagtccaacggcaccatcatccacgtgaagggcaagcacctgtgtccttctccactgttccccggacctagcaagcctttttgggtgctggtggtggttggtggagtcctggcttgctatagcttgctagtaacagtggcctttattattttctgggtgaggagtaagaggagcaggctcctgcacagtgactacatgaacatgactccccgccgccccgggcccacccgcaagcattaccagccctatgccccaccacgcgacttcgcagcctatcgctccctgagagtgaagttcagcaggagcgcagacgcccccgcgtaccagcagggccagaaccagctctataacgagctcaatctaggacgaagagaggagtacgatgttttggacaagagacgtggccgggaccctgagatggggggaaagccgcagagaaggaagaaccctcaggaaggcctgtacaatgaactgcagaaagataagatggcggaggcctacagtgagattgggatgaaaggcgagcgccggaggggcaaggggcacgatggcctttaccagggtctcagtacagccaccaaggacacctacgacgcccttcacatgcaggccctgccccctcgctaa

SEQ ID NO: 110 - protein, 482 aa, synthetic construct
MKHLWFFLLLVAAPRWVLSDIQMTQTTSSLSASLGDRVTISCRASQDISKYLNWYQQKPDGTVKLLIYHTSRLHSGVPSRFSGSGSGTDYSLTISNLEQEDIATYFCQQGNTLPYTFGGGTKLEITGGGGSGGGGSGGGGSEVKLQESGPGLVAPSQSLSVTCTVSGVSLPDYGVSWIRQPPRKGLEWLGVIWGSETTYYNSALKSRLTIIKDNSKSQVFLKMNSLQTDDTAIYYCAKHYYYGGSYAMDYWGQGTSVTVSSIEVMYPPPYLDNEKSNGTIIHVKGKHLCPSPLFPGPSKPFWVLVVVGGVLACYSLLVTVAFIIFWVRSKRSRLLHSDYMNMTPRRPGPTRKHYQPYAPPRDFAAYRSLRVKFSRSADAPAYQQGQNQLYNELNLGRREEYDVLDKRRGRDPEMGGKPQRRKNPQEGLYNELQKDKMAEAYSEIGMKGERRRGKGHDGLYQGLSTATKDTYDALHMQALPPR

SEQ ID NO: 111 - protein, 482 aa, synthetic construct
MKHLWFFLLLVAAPRWVLSDIQMTQTTSSLSASLGDRVTISCRASQDISKYLNWYQQKPDGTVKLLIYHTSRLHSGVPDRFDGDGSGTDYSLTISNLEQEDIATYFCQQGNTLPYTFGGGTKLEITGGGGSGGGGSGGGGSEVKLQESGPGLVAPSQSLSVTCTVSGVSLPDYGVSWIRQPPRKGLEWLGVIWGSETTYYNSALKSRLTIIKDNSKSQVFLKMNSLQTDDTAIYYCAKHYYYGGSYAMDYWGQGTSVTVSSIEVMYPPPYLDNEKSNGTIIHVKGKHLCPSPLFPGPSKPFWVLVVVGGVLACYSLLVTVAFIIFWVRSKRSRLLHSDYMNMTPRRPGPTRKHYQPYAPPRDFAAYRSLRVKFSRSADAPAYQQGQNQLYNELNLGRREEYDVLDKRRGRDPEMGGKPQRRKNPQEGLYNELQKDKMAEAYSEIGMKGERRRGKGHDGLYQGLSTATKDTYDALHMQALPPR

SEQ ID NO: 112 - protein, 482 aa, synthetic construct
MKHLWFFLLLVAAPRWVLSDIQMTQTTSSLSASLGDRVTISCRASQDISKYLNWYQQKPDGTVKLLIYHTSRLHSGVPSRFSGSGSGTEYELEISNLEQEDIATYFCQQGNTLPYTFGGGTKLEITGGGGSGGGGSGGGGSEVKLQESGPGLVAPSQSLSVTCTVSGVSLPDYGVSWIRQPPRKGLEWLGVIWGSETTYYNSALKSRLTIIKDNSKSQVFLKMNSLQTDDTAIYYCAKHYYYGGSYAMDYWGQGTSVTVSSIEVMYPPPYLDNEKSNGTIIHVKGKHLCPSPLFPGPSKPFWVLVVVGGVLACYSLLVTVAFIIFWVRSKRSRLLHSDYMNMTPRRPGPTRKHYQPYAPPRDFAAYRSLRVKFSRSADAPAYQQGQNQLYNELNLGRREEYDVLDKRRGRDPEMGGKPQRRKNPQEGLYNELQKDKMAEAYSEIGMKGERRRGKGHDGLYQGLSTATKDTYDALHMQALPPR

SEQ ID NO: 113 - protein, 482 aa, synthetic construct
MKHLWFFLLLVAAPRWVLSDIQMTQTTSSLSASLGDRVTISCRASQDISKYLNWYQQKPDGTVKLLIYHTSRLHSGVPSRFDGDGSGTDYDLTISNLEQEDIATYFCQQGNTLPYTFGGGTKLEITGGGGSGGGGSGGGGSEVKLQESGPGLVAPSQSLSVTCTVSGVSLPDYGVSWIRQPPRKGLEWLGVIWGSETTYYNSALKSRLTIIKDNSKSQVFLKMNSLQTDDTAIYYCAKHYYYGGSYAMDYWGQGTSVTVSSIEVMYPPPYLDNEKSNGTIIHVKGKHLCPSPLFPGPSKPFWVLVVVGGVLACYSLLVTVAFIIFWVRSKRSRLLHSDYMNMTPRRPGPTRKHYQPYAPPRDFAAYRSLRVKFSRSADAPAYQQGQNQLYNELNLGRREEYDVLDKRRGRDPEMGGKPQRRKNPQEGLYNELQKDKMAEAYSEIGMKGERRRGKGHDGLYQGLSTATKDTYDALHMQALPPR

SEQ ID NO: 114 - protein, 482 aa, synthetic construct
MKHLWFFLLLVAAPRWVLSDIQMTQTTSSLSASLGDRVTISCRASQDISKYLNWYQQKPDGTVKLLIYHTSRLHSGVPSRFDGSGDGTDYDLTISNLEQEDIATYFCQQGNTLPYTFGGGTKLEITGGGGSGGGGSGGGGSEVKLQESGPGLVAPSQSLSVTCTVSGVSLPDYGVSWIRQPPRKGLEWLGVIWGSETTYYNSALKSRLTIIKDNSKSQVFLKMNSLQTDDTAIYYCAKHYYYGGSYAMDYWGQGTSVTVSSIEVMYPPPYLDNEKSNGTIIHVKGKHLCPSPLFPGPSKPFWVLVVVGGVLACYSLLVTVAFIIFWVRSKRSRLLHSDYMNMTPRRPGPTRKHYQPYAPPRDFAAYRSLRVKFSRSADAPAYQQGQNQLYNELNLGRREEYDVLDKRRGRDPEMGGKPQRRKNPQEGLYNELQKDKMAEAYSEIGMKGERRRGKGHDGLYQGLSTATKDTYDALHMQALPPR

SEQ ID NO: 115 - protein, 482 aa, synthetic construct
MKHLWFFLLLVAAPRWVLSDIQMTQTTSSLSASLGDRVTISCRASQDISKYLNWYQQKPDGTVKLLIYHTSRLHSGVPSRFDGDGDGTDYDLTISNLEQEDIATYFCQQGNTLPYTFGGGTKLEITGGGGSGGGGSGGGGSEVKLQESGPGLVAPSQSLSVTCTVSGVSLPDYGVSWIRQPPRKGLEWLGVIWGSETTYYNSALKSRLTIIKDNSKSQVFLKMNSLQTDDTAIYYCAKHYYYGGSYAMDYWGQGTSVTVSSIEVMYPPPYLDNEKSNGTIIHVKGKHLCPSPLFPGPSKPFWVLVVVGGVLACYSLLVTVAFIIFWVRSKRSRLLHSDYMNMTPRRPGPTRKHYQPYAPPRDFAAYRSLRVKFSRSADAPAYQQGQNQLYNELNLGRREEYDVLDKRRGRDPEMGGKPQRRKNPQEGLYNELQKDKMAEAYSEIGMKGERRRGKGHDGLYQGLSTATKDTYDALHMQALPPR

SEQ ID NO: 116 - protein, 482 aa, synthetic construct
MKHLWFFLLLVAAPRWVLSDIQMTQTTSSLSASLGDRVTISCRASQDISKYLNWYQQKPDGTVKLLIYHTSRLHSGVPSRFEGEGEGTEYELTISNLEQEDIATYFCQQGNTLPYTFGGGTKLEITGGGGSGGGGSGGGGSEVKLQESGPGLVAPSQSLSVTCTVSGVSLPDYGVSWIRQPPRKGLEWLGVIWGSETTYYNSALKSRLTIIKDNSKSQVFLKMNSLQTDDTAIYYCAKHYYYGGSYAMDYWGQGTSVTVSSIEVMYPPPYLDNEKSNGTIIHVKGKHLCPSPLFPGPSKPFWVLVVVGGVLACYSLLVTVAFIIFWVRSKRSRLLHSDYMNMTPRRPGPTRKHYQPYAPPRDFAAYRSLRVKFSRSADAPAYQQGQNQLYNELNLGRREEYDVLDKRRGRDPEMGGKPQRRKNPQEGLYNELQKDKMAEAYSEIGMKGERRRGKGHDGLYQGLSTATKDTYDALHMQALPPR

SEQ ID NO: 117 - DNA, 138 bp, synthetic construct
  source 1..138: mol_type = other DNA
accaccactcctgcacctaggccacccacgcctgccccaactattgcatcccagcctctgtctctgcgccccgaagcctgtcggcctgcagctggaggcgccgtgcacactcggggcctcgacttcgcatgtgatatc

SEQ ID NO: 118 - DNA, 339 bp, synthetic construct
  source 1..339: mol_type = other DNA
ctgcgcgtgaagttctccaggagcgctgacgcgcccgcttacaagcaggggcagaatcagctgtacaacgaattgaacctcgggcgtcgcgaggagtatgacgtcctcgacaagcgaaggggccgggacccggaaatgggaggcaagccacgcaggaagaatccccaagagggactgtataacgagctccagaaggacaaaatggctgaagcctacagcgaaattggtatgaaaggggagcgcagaagaggaaaggggcatgacgggctctaccagggattgagcactgccaccaaagacacctatgacgctctgcacatgcaagctctgccacctaga

SEQ ID NO: 119 - protein, 46 aa, synthetic construct
TTTPAPRPPTPAPTIASQPLSLRPEACRPAAGGAVHTRGLDFACDI

SEQ ID NO: 120 - protein, 113 aa, synthetic construct
LRVKFSRSADAPAYKQGQNQLYNELNLGRREEYDVLDKRRGRDPEMGGKPRRKNPQEGLYNELQKDKMAEAYSEIGMKGERRRGKGHDGLYQGLSTATKDTYDALHMQALPPR